European Patent Specification EP 3 962 491 B1, published August 6, 2025. Title: Intracellular delivery of anti-KRAS antibodies formulated into nanocapsules. Applicant: USC UNIVERSIDADE DE SANTIAGO DE COMPOSTELA. The sequence listing filed with the application follows.

SEQUENCE LISTING (50 sequences)

SEQ ID NO: 1 - protein, 9 aa, Artificial Sequence
  Synthetic sequence
CGNKRTRGC

SEQ ID NO: 2 - protein, 7 aa, Artificial Sequence
  Synthetic sequence
CGNKRTR

SEQ ID NO: 3 - protein, 9 aa, Artificial Sequence
  Synthetic sequence
CGNKRTRGC

SEQ ID NO: 4 - protein, 9 aa, Artificial Sequence
  Synthetic sequence
CRNGRGPDC

SEQ ID NO: 5 - protein, 9 aa, Artificial Sequence
  Synthetic sequence
CRGDKGPDC

SEQ ID NO: 6 - protein, 9 aa, Artificial Sequence
  Synthetic sequence
CRGDRGPDC

SEQ ID NO: 7 - protein, 7 aa, Artificial Sequence
  Synthetic sequence
RPARPAR

SEQ ID NO: 8 - protein, 9 aa, Artificial Sequence
  Synthetic sequence
CKRGARSTC

SEQ ID NO: 9 - protein, 9 aa, Artificial Sequence
  Synthetic sequence
AKRGARSTA

SEQ ID NO: 10 - protein, 462 aa, Antibody polypeptide
  Antibody polypeptide from hybridoma DSM ACC3358
MGWSYIILFLVATATGVHSQVQLQQSGAELVKPGASVKLSCKASGYTFTSYYMYWVKQRPGQGLEWIGEINPSNGGTNFNEKFKSKATLTVDKSSGTAYMQLSSLTSEDSAIYYCTRGGYGYWGQGTTLTVSSAKTTPPSVYPLAPGSAAQTNSMVTLGCLVKGYFPEPVTVTWNSGSLSSGVHTFPAVLQSDLYTLSSSVTVPSSTWPSETVTCNVAHPASSTKVDKKIVPRDCGCKPCICTVPEVSSVFIFPPKPKDVLTITLTPKVTCVVVDISKDDPEVQFSWFVDDVEVHTAQTQPREEQFNSTFRSVSELPIMHQDWLNGKEFKCRVNSAAFPAPIEKTISKTKGRPKAPQVYTIPPPKEQMAKDKVSLTCMITDFFPEDITVEWQWNGQPAENYKNTQPIMDTDGSYFVYSKLNVQKSNWEAGNTFTCSVLHEGLHNHHTEKSLSHSPGKLIGHT

SEQ ID NO: 11 - protein, 9 aa, Artificial Sequence
  Synthetic sequence
CDCRGDCFC

SEQ ID NO: 12 - protein, 9 aa, Artificial Sequence
  Synthetic sequence
CRGDLASLC

SEQ ID NO: 13 - protein, 4 aa, Artificial Sequence
  Synthetic sequence
RGDK

SEQ ID NO: 14 - protein, 4 aa, Artificial Sequence
  Synthetic sequence
VRGD

SEQ ID NO: 15 - protein, 11 aa, Artificial Sequence
  Synthetic sequence
KLWVLPKGGGC

SEQ ID NO: 16 - protein, 11 aa, Artificial Sequence
  Synthetic sequence
KLWVLPKGGGC

SEQ ID NO: 17 - protein, 239 aa, Antibody polypeptide
  Antibody polypeptide from hybridoma DSM ACC3358
MRCSLQFLGVLMFWISGVSGDIVITQDELSNPVISGESVSISCRSSKSLLYKDGKTYLNWFLQRPGQSPQLLIYLMSTRASGVSDRFSGSGSGTDFTLEISRVKAEDVGVYYCQQVVEYPRTFGSGTKLEIKRADAAPTVSIFPPSSEQLTSGGASVVCFLNNFYPKDINVKWKIDGSERQNGVLNSWTDQDSKDSTYSMSSTLTLTKDEYERHNSYTCEATHKTSTSPIVKSFNRNEC

SEQ ID NO: 18 - protein, 9 aa, Artificial Sequence
  Synthetic sequence
CPGPEGAGC

SEQ ID NO: 19 - protein, 5 aa, Artificial Sequence
  Synthetic sequence
CREKA

SEQ ID NO: 20 - protein, 29 aa, Artificial Sequence
  Synthetic sequence
YTIWMPENPRPGTPCDIFTNSRGKRASNG

SEQ ID NO: 21 - protein, 11 aa, Artificial Sequence
  Synthetic sequence
LGASWHRPDKG

SEQ ID NO: 22 - protein, 5 aa, Artificial Sequence
  Synthetic sequence
DEVDG

SEQ ID NO: 23 - protein, 6 aa, Artificial Sequence
  Synthetic sequence
PLGLAG

SEQ ID NO: 24 - protein, 10 aa, Artificial Sequence
  Synthetic sequence
IAGEDGDEFG

SEQ ID NO: 25 - protein, 12 aa, Artificial Sequence
  Synthetic sequence
RRRRRRRRGRGD

SEQ ID NO: 26 - protein, 9 aa, Artificial Sequence
  Synthetic sequence
CRGDKGPDC

SEQ ID NO: 27 - protein, 9 aa, Artificial Sequence
  Synthetic sequence
CGNKRTRGC

SEQ ID NO: 28 - protein, 9 aa, Artificial Sequence
  Synthetic sequence
CGNKRTRGC

SEQ ID NO: 29 - protein, 9 aa, Artificial Sequence
  Synthetic sequence
CKRGARSTC

SEQ ID NO: 30 - protein, 9 aa, Artificial Sequence
  Synthetic peptide
AKRGARSTA

SEQ ID NO: 31 - protein, 9 aa, Artificial Sequence
  Synthetic sequence
CRNGRGPDC

SEQ ID NO: 32 - protein, 31 aa, Artificial Sequence
  Synthetic sequence
KDEPQRRSARLSAKPAPPKPEPKPKKAPAKK

SEQ ID NO: 33 - protein, 6 aa, Artificial Sequence
  Antibody polypeptide from hybridoma DSM ACC3359
SGYYWN

SEQ ID NO: 34 - protein, 16 aa, Artificial Sequence
  Antibody polypeptide from hybridoma DSM ACC3359
YIGYDGTNNYNPSLKN

SEQ ID NO: 35 - protein, 4 aa, Artificial Sequence
  Antibody polypeptide from hybridoma DSM ACC3359
LWDY

SEQ ID NO: 36 - protein, 16 aa, Artificial Sequence
  Antibody polypeptide from hybridoma DSM ACC3359
RSSQTIVHGNGNTYLE

SEQ ID NO: 37 - protein, 7 aa, Artificial Sequence
  Antibody polypeptide from hybridoma DSM ACC3359
TVSNRFS

SEQ ID NO: 38 - protein, 9 aa, Artificial Sequence
  Antibody polypeptide from hybridoma DSM ACC3359
FQGSHAPYT

SEQ ID NO: 39 - protein, 188 aa, Human KRAS gene [sequence omitted]

SEQ ID NO: 40 - protein, 12 aa, Artificial Sequence
  Synthetic sequence
KLVVVGAVGVGK

SEQ ID NO: 41 - protein, 12 aa, Artificial Sequence
  Synthetic sequence
KLVVVGADGVGK

SEQ ID NO: 42 - protein, 12 aa, Artificial Sequence
  Synthetic sequence
KLVVVGACGVGK

SEQ ID NO: 43 - protein, 467 aa, Antibody polypeptide heavy-chain region
  Antibody polypeptide from hybridoma DSM ACC3359
MKVLSLLYLLTAIPGILSDIQLQESGPGLVKPSQSLSLTCSVTGYSITSDYYWNWIRQFPGNKLEWMGYIGYDGTNNYNPSLKNRISITRDTSKNQFFLKLNSVTAEDTATYYCARLWDYWGQGTTLTVSSAKTTPPSVYPLAPGCGDTTGSSVTLGCLVKGYFPESVTVTWNSGSLSSSVHTFPALLQSGLYTMSSSVTVPSSTWPSQTVTCSVAHPASSTTVDKKLEPSGPISTINPCPPCKECHKCPAPNLEGGPSVFIFPPNIKDVLMISLTPKVTCVVVDVSEDDPDVQISWFVNNVEVHTAQTQTHREDYNSTIRVVSTLPIQHQDWMSGKEFKCKVNNKDLPSPIERTISKIKGLVRAPQVYILPPPAEQLSRKDVSLTCLVVGFNPGDISVEWTSNGHTEENYKDTAPVLDSDGSYFIYSKLNMKTSKWEKTDSFSCNVRHEGLKNYYLKKTISRSPGK

SEQ ID NO: 44 - protein, 238 aa, Antibody polypeptide light-chain region
  Antibody polypeptide from hybridoma DSM ACC3359
MKLPVRLLVLMFWIPASSSDVLMTQTPLSLPVSLGDQASISCRSSQTIVHGNGNTYLEWYLQKPGQSPKLLIYTVSNRFSGVPDRFSGSGSGTDFTLKISRVEAEDLGVYYCFQGSHAPYTFGGGTKLEIKRADAAPTVSIFPPSSEQLTSGGASVVCFLNNFYPKDINVKWKIDGSERQNGVLNSWTDQDSKDSTYSMSSTLTLTKDEYERHNSYTCEATHKTSTSPIVKSFNRNEC

SEQ ID NO: 45 - protein, 5 aa, Artificial Sequence
  Antibody polypeptide from hybridoma DSM ACC3358
SYYMY

SEQ ID NO: 46 - protein, 17 aa, Artificial Sequence
  Antibody polypeptide from hybridoma DSM ACC3358
EINPSNGGTNFNEKFKS

SEQ ID NO: 47 - protein, 5 aa, Artificial Sequence
  Hybridoma DSM ACC3358Antibody polypeptide from hybridoma DSM ACC3358
GGYGY

SEQ ID NO: 48 - protein, 16 aa, Artificial Sequence
  Antibody polypeptide from hybridoma DSM ACC3358
RSSKSLLYKDGKTYLN

SEQ ID NO: 49 - protein, 7 aa, Artificial Sequence
  Antibody polypeptide from hybridoma DSM ACC3358
LMSTRAS

SEQ ID NO: 50 - protein, 9 aa, Artificial Sequence
  Antibody polypeptide from hybridoma DSM ACC3358
QQVVEYPRT